European Patent Specification EP 3 650 540 B1, published April 16, 2025. Title: Target Specific CRISPR variants. Applicant: ToolGen Incorporated. The sequence listing filed with the application follows.

SEQUENCE LISTING (11 sequences)

SEQ ID NO: 1 - protein, 1368 aa, Streptococcus pyogenes [sequence omitted]

SEQ ID NO: 2 - protein, 87 aa, Streptococcus pyogenes
FEENPINASGVDAKAILSARLSKSRRLENLIAQLPGEKKNGLFGNLIALSLGLTPNFKSNFDLAEDAKLQLSKDTYDDDLDNLLAQI

SEQ ID NO: 3 - protein, 79 aa, Streptococcus pyogenes
PLSASMIKRYDEHHQDLTLLKALVRQQLPEKYKEIFFDQSKNGYAGYIDGGASQEEFYKFIKPILEKMDGTEELLVKLN

SEQ ID NO: 4 - protein, 103 aa, Streptococcus pyogenes
KHSLLYEYFTVYNELTKVKYVTEGMRKPAFLSGEQKKAIVDLLFKTNRKVTVKQLKEDYFKKIECFDSVEISGVEDRFNASLGTYHDLLKIIKDKDFLDNEEN

SEQ ID NO: 5 - protein, 21 aa, Streptococcus pyogenes
TILDFLKSDGFANRNFMQLIH

SEQ ID NO: 6 - protein, 22 aa, Streptococcus pyogenes
MDKKYSIGLDIGTNSVGWAVIT

SEQ ID NO: 7 - protein, 40 aa, Streptococcus pyogenes
PAIKKGILQTVKVVDELVKVMGRHKPENIVIEMARENQTT

SEQ ID NO: 8 - protein, 115 aa, Streptococcus pyogenes
QITKHVAQILDSRMNTKYDENDKLIREVKVITLKSKLVSDFRKDFQFYKVREINNYHHAHDAYLNAVVGTALIKKYPKLESEFVYGDYKVYDVRKMIAKSEQEIGKATAKYFFYS

SEQ ID NO: 9 - protein, 126 aa, Streptococcus pyogenes
KNSRERMKRIEEGIKELGSQILKEHPVENTQLQNEKLYLYYLQNGRDMYVDQELDINRLSDYDVDHIVPQSFLKDDSIDNKVLTRSDKNRGKSDNVPSEEVVKKMKNYWRQLLNAKLITQRKFDNL

SEQ ID NO: 10 - protein, 41 aa, Streptococcus pyogenes
EVQTGGFSKESILPKRNSDKLIARKKDWDPKKYGGFDSPTV

SEQ ID NO: 11 - protein, 1368 aa, Artificial Sequence
  Streptococcus pyogenes Cas9 variant
MDKKYSIGLDIGTNSVGWAVITDEYKVPSKKFKVLGNTDRHSIKKNLIGALLFDSGETAEATRLKRTARRRYTRRKNRICYLQEIFSNEMAKVDDSFFHRLEESFLVEEDKKHERHPIFGNIVDEVAYHEKYPTIYHLRKKLVDSTDKADLRLIYLALAHMIKFRGHFLIEGDLNPDNSDVDKLFIQLVQTYNQLFEENPINASGVDAKAILSARLSKSRRLENLIAQLPGEKKNGLFGNLIALSLGLTPNFKSNFDLAEDAKLQLSKDTYDDDLDNLLAQIGDQYADLFLAAKNLSDAILLSDILRVNTEITKAPLSASMIKRYDEHHQDLTLLKALVRQQLPEKYKEIFFDQSKNGYAGYIDGGASQEEFYKFIKPILEKMDGTEELLVKLNREDLLRKQRTFDNGSIPHQIHLGELHAILRRQEDFYPFLKDNREKIEKILTFRIPYYVGPLARGNSRFAWMTRKSEETITPWNFEEVVDKGASAQSFIERMTNFDKNLPNEKVLPKHSLLYEYFTVYNELTKVKYVTEGMRKPASLSGEQKKAIVDLLFKTNRKVTVKQLKEDYFKKIECFDSVEISGVEDRFNASLGTYHDLLKIIKDKDFLDNEENEDILEDIVLTLTLFEDREMIEERLKTYAHLFDDKVMKQLKRRRYTGWGRLSRKLINGIRDKQSGKTILDFLKSDGFANRNFMQLIHDDSLTFKEDIQKAQVSGQGDSLHEHIANLAGSPAIKKGILQTVKVVDELVKVMGRHKPENIVIEIARENQTTQKGQKNSRERMKRIEEGIKELGSQILKEHPVENTQLQNEKLYLYYLQNGRDMYVDQELDINRLSDYDVDHIVPQSFLKDDSIDNKVLTRSDKNRGKSDNVPSEEVVKKMKNYWRQLLNANLITQRKFDNLTKAERGGLSELDKAGFIKRQLVETRQITKHVAQILDSRMNTKYDENDKLIREVKVITLKSKLVSDFRKDFQFYKVREINNYHHAHDAYLNAVVGTALIKKYPKLESEFVYGDYKVYDVRKMIAKSEQEIGKATAKYFFYSNIMNFFKTEITLANGEIRKRPLIETNGETGEIVWDKGRDFATVRKVLSMPQVNIVKKTEVQTGGFSKESILPKRNSDKLIARKKDWDPKKYGGFDSPTVAYSVLVVAKVEKGKSKKLKSVKELLGITIMERSSFEKNPIDFLEAKGYKEVKKDLIIKLPKYSLFELENGRKRMLASAGELQKGNELALPSKYVNFLYLASHYEKLKGSPEDNEQKQLFVEQHKHYLDEIIEQISEFSKRVILADANLDKVLSAYNKHRDKPIREQAENIIHLFTLTNLGAPAAFKYFDTTIDRKRYTSTKEVLDATLIHQSITGLYETRIDLSQLGGD